European Patent Specification EP 3 565 887 B1, published July 16, 2025. Title: Methods for Generating Skeletal Muscle Progenitor Cells. Applicant: Pyle, April D Hicks, Michael R. The sequence listing filed with the application follows.

SEQUENCE LISTING (43 sequences)

SEQ ID NO: 1 - DNA, 22 bp, Artificial Sequence
  synthetic nucleic acid
cgcccccggtttctataaattg

SEQ ID NO: 2 - DNA, 20 bp, Artificial Sequence
  synthetic nucleic acid
aagaagatgcggctgactgt

SEQ ID NO: 3 - DNA, 21 bp, Artificial Sequence
  synthetic nucleic acid
agctcggcggtgtttttatca

SEQ ID NO: 4 - DNA, 21 bp, Artificial Sequence
  synthetic nucleic acid
ctgcacaggatcttggagacg

SEQ ID NO: 5 - DNA, 20 bp, Artificial Sequence
  synthetic nucleic acid
ctggccaaaaatgtgagcct

SEQ ID NO: 6 - DNA, 20 bp, Artificial Sequence
  synthetic nucleic acid
tagggttgggctgggaattg

SEQ ID NO: 7 - DNA, 20 bp, Artificial Sequence
  synthetic nucleic acid
ttaaccacaaatcaggccgg

SEQ ID NO: 8 - DNA, 22 bp, Artificial Sequence
  synthetic nucleic acid
caaagtgctggcagtctgaatg

SEQ ID NO: 9 - DNA, 20 bp, Artificial Sequence
  synthetic nucleic acid
agatgtgtctgtggccttcc

SEQ ID NO: 10 - DNA, 20 bp, Artificial Sequence
  synthetic nucleic acid
agctggcttcctagcatcag

SEQ ID NO: 11 - DNA, 24 bp, Artificial Sequence
  synthetic nucleic acid
tgcccttgttaattaccggagcga

SEQ ID NO: 12 - DNA, 23 bp, Artificial Sequence
  synthetic nucleic acid
tatgcaggagccgtcgtagaagt

SEQ ID NO: 13 - DNA, 21 bp, Artificial Sequence
  synthetic nucleic acid
ggaagaaacgcagagggatca

SEQ ID NO: 14 - DNA, 21 bp, Artificial Sequence
  synthetic nucleic acid
caagcgtcgcaattcagaaag

SEQ ID NO: 15 - DNA, 20 bp, Artificial Sequence
  synthetic nucleic acid
cctgtcatccccgtctacac

SEQ ID NO: 16 - DNA, 19 bp, Artificial Sequence
  synthetic nucleic acid
cacatggagtccgccgtaa

SEQ ID NO: 17 - DNA, 21 bp, Artificial Sequence
  synthetic nucleic acid
acctattggaggcgactttcc

SEQ ID NO: 18 - DNA, 20 bp, Artificial Sequence
  synthetic nucleic acid
tccttccaaaggctgctctg

SEQ ID NO: 19 - DNA, 20 bp, Artificial Sequence
  synthetic nucleic acid
ccttctggagcaggacagaa

SEQ ID NO: 20 - DNA, 23 bp, Artificial Sequence
  synthetic nucleic acid
caaagcaaagtttattgcatgtg

SEQ ID NO: 21 - DNA, 21 bp, Artificial Sequence
  synthetic nucleic acid
attgcttcgtggtggactcaa

SEQ ID NO: 22 - DNA, 21 bp, Artificial Sequence
  synthetic nucleic acid
ggccatgtcttcgatcctgtc

SEQ ID NO: 23 - DNA, 22 bp, Artificial Sequence
  synthetic nucleic acid
gtagttgtctgctttgagcctg

SEQ ID NO: 24 - DNA, 20 bp, Artificial Sequence
  synthetic nucleic acid
ttgtaggggttgacggtgac

SEQ ID NO: 25 - DNA, 22 bp, Artificial Sequence
  synthetic nucleic acid
aatgcaagtgctattccagagg

SEQ ID NO: 26 - DNA, 22 bp, Artificial Sequence
  synthetic nucleic acid
acagacagcttgtgttcttgtt

SEQ ID NO: 27 - DNA, 22 bp, Artificial Sequence
  synthetic nucleic acid
ctgaatttctcaaccgacaaca

SEQ ID NO: 28 - DNA, 23 bp, Artificial Sequence
  synthetic nucleic acid
catatctgttttgtagccaggag

SEQ ID NO: 29 - DNA, 20 bp, Artificial Sequence
  synthetic nucleic acid
gttgtccgcctctgtcttct

SEQ ID NO: 30 - DNA, 20 bp, Artificial Sequence
  synthetic nucleic acid
tctatccacgtgcctacagc

SEQ ID NO: 31 - DNA, 20 bp, Artificial Sequence
  synthetic nucleic acid
cgagagctacacgttcacgg

SEQ ID NO: 32 - DNA, 21 bp, Artificial Sequence
  synthetic nucleic acid
gggtgtcgagggaaaaatagg

SEQ ID NO: 33 - DNA, 19 bp, Artificial Sequence
  synthetic nucleic acid
ggagctggctacttctcgc

SEQ ID NO: 34 - DNA, 21 bp, Artificial Sequence
  synthetic nucleic acid
gggtgtcgagggaaaaatagg

SEQ ID NO: 35 - DNA, 21 bp, Artificial Sequence
  synthetic nucleic acid
aaaagacagctacgtgggtga

SEQ ID NO: 36 - DNA, 22 bp, Artificial Sequence
  synthetic nucleic acid
gccatgttctatcgggtacttc

SEQ ID NO: 37 - DNA, 22 bp, Artificial Sequence
  synthetic nucleic acid
tcctggctaacgacaaatacga

SEQ ID NO: 38 - DNA, 20 bp, Artificial Sequence
  synthetic nucleic acid
tttcccggccaccataaagg

SEQ ID NO: 39 - DNA, 20 bp, Artificial Sequence
  synthetic nucleic acid
taaggcgccctcaagatcaa

SEQ ID NO: 40 - DNA, 20 bp, Artificial Sequence
  synthetic nucleic acid
gagcttcttcactgccacac

SEQ ID NO: 41 - DNA, 23 bp, Artificial Sequence
  synthetic nucleic acid
tcgtacttcccattgcgatagaa

SEQ ID NO: 42 - DNA, 21 bp, Artificial Sequence
  Synthetic nucleic acid
ctgacaagcacaagactgacc

SEQ ID NO: 43 - DNA, 21 bp, Artificial Sequence
  Synthetic nucleic acid
ctgctgagcacgtagttaggg